European Patent Specification EP 3 772 927 B1, published January 15, 2025. Title: GENETICALLY MODIFIED NON-HUMAN ANIMALS FOR GENERATING THERAPEUTIC ANTIBODIES AGAINST PEPTIDE-MHC COMPLEXES, METHODS OF MAKING AND USES THEREOF. Applicant: Regeneron Pharmaceuticals, Inc. Murphy, Andrew J. The sequence listing filed with the application follows.

SEQUENCE LISTING (29 sequences)

SEQ ID NO: 1 - protein, 5 aa, Artificial Sequence
  Linker sequence
GSGGS

SEQ ID NO: 2 - protein, 4 aa, Artificial Sequence
  Linker sequence
GGGS

SEQ ID NO: 3 - protein, 4 aa, Artificial Sequence
  Linker sequence
GGSG

SEQ ID NO: 4 - protein, 5 aa, Artificial Sequence
  Linker sequence
GGSGG

SEQ ID NO: 5 - protein, 5 aa, Artificial Sequence
  Linker sequence
GSGSG

SEQ ID NO: 6 - protein, 5 aa, Artificial Sequence
  Linker sequence
GSGGG

SEQ ID NO: 7 - protein, 5 aa, Artificial Sequence
  Linker sequence
GGGSG

SEQ ID NO: 8 - protein, 5 aa, Artificial Sequence
  Linker sequence
GSSSG

SEQ ID NO: 9 - protein, 15 aa, Artificial Sequence
  Linker sequence
GCGASGGGGSGGGGS

SEQ ID NO: 10 - protein, 15 aa, Artificial Sequence
  Linker sequence
GCGASGGGGSGGGGS

SEQ ID NO: 11 - protein, 10 aa, Artificial Sequence
  Linker sequence
GGGGSGGGGS

SEQ ID NO: 12 - protein, 15 aa, Artificial Sequence
  Linker sequence
GGGASGGGGSGGGGS

SEQ ID NO: 13 - protein, 15 aa, Artificial Sequence
  Linker sequence
GGGGSGGGGSGGGGS

SEQ ID NO: 14 - protein, 10 aa, Artificial Sequence
  Linker sequence
GGGASGGGGS

SEQ ID NO: 15 - protein, 15 aa, Artificial Sequence
  Linker sequence
GGGGSGGGGSGGGGS

SEQ ID NO: 16 - protein, 20 aa, Artificial Sequence
  Linker sequence
GGGGSGGGGSGGGGSGGGGS

SEQ ID NO: 17 - DNA, 1230 bp, Artificial Sequence
  GCGGS+G4Sx2-hB2m-G4Sx4-hHLA-A2 ecto Y108C
ggatgcggaggtagtgggggaggtggctccgggggagggggatccatacagcggactccaaagatccaggtgtatagtcgccaccccgcagagaatggaaagtccaacttccttaactgttatgtgagcggatttcacccttcagacatagaggtagaccttctgaaaaacggagagagaatagagaaggtagagcatagtgatctttctttttccaaggactggagcttctacctcctgtactataccgagtttacacccactgagaaggatgagtacgcatgccgcgtgaaccacgtaaccctttctcaaccaaagattgtaaaatgggacagagacatgggtggcggcggtagcggcgggggcggaagcggcggaggaggctccggtgggggtggttcagggtcccattctatgagatatttttttacaagcgtgagccggcctgggaggggggagccccggtttatcgctgtggggtacgtggatgatactcaattcgtgcggttcgactctgacgccgcctcacagcgcatggagcctagggcaccctggattgaacaggagggcccggaatactgggacggcgaaacccgcaaggtaaaagcgcacagccagacgcatagggtggatctgggcaccctgcggggctgttataaccagtcagaggctggctcacacactgtacagcggatgtatggttgtgacgtcggttccgattggagatttcttcgcggctaccaccaatacgcctacgatggcaaggactacatcgcactgaaggaagatttgagatcttggaccgcggcggatatggcagcacagactaccaaacacaagtgggaagctgctcatgtggcagaacagctccgcgcctatctggagggcacttgcgtcgagtggttgcggagatacctggagaatgggaaagaaacactgcagcggaccgatgcacctaaaacacatatgacgcaccacgctgtgtccgaccacgaggcaacactccggtgttgggcactcagcttctaccctgctgaaataacgctgacctggcagcgcgacggcgaagatcagacgcaggacacagagcttgttgaaactcgccctgctggcgacggcaccttccaaaaatgggcagcagtagtcgtcccctccggacaggaacagcggtatacttgccacgtgcagcatgaaggtctccccaagcccctcactctgagatgggagccg

SEQ ID NO: 18 - protein, 410 aa, Artificial Sequence
  GCGGS+G4Sx2-hB2m-G4Sx4-hHLA-A2 ecto Y108C
GCGGSGGGGSGGGGSIQRTPKIQVYSRHPAENGKSNFLNCYVSGFHPSDIEVDLLKNGERIEKVEHSDLSFSKDWSFYLLYYTEFTPTEKDEYACRVNHVTLSQPKIVKWDRDMGGGGSGGGGSGGGGSGGGGSGSHSMRYFFTSVSRPGRGEPRFIAVGYVDDTQFVRFDSDAASQRMEPRAPWIEQEGPEYWDGETRKVKAHSQTHRVDLGTLRGCYNQSEAGSHTVQRMYGCDVGSDWRFLRGYHQYAYDGKDYIALKEDLRSWTAADMAAQTTKHKWEAAHVAEQLRAYLEGTCVEWLRRYLENGKETLQRTDAPKTHMTHHAVSDHEATLRCWALSFYPAEITLTWQRDGEDQTQDTELVETRPAGDGTFQKWAAVVVPSGQEQRYTCHVQHEGLPKPLTLRWEP

SEQ ID NO: 19 - DNA, 1511 bp, Artificial Sequence
  GCGGS+G4Sx2-hB2m-G4Sx4-HLA-A2 Y108C (G4S)4
ctcctcatgggaacgctcggcatagtgggatgcggaggtagtgggggaggtggctccgggggagggggatccatacagcggactccaaagatccaggtgtatagtcgccaccccgcagagaatggaaagtccaacttccttaactgttatgtgagcggatttcacccttcagacatagaggtagaccttctgaaaaacggagagagaatagagaaggtagagcatagtgatctttctttttccaaggactggagcttctacctcctgtactataccgagtttacacccactgagaaggatgagtacgcatgccgcgtgaaccacgtaaccctttctcaaccaaagattgtaaaatgggacagagacatgggtggcggcggtagcggcgggggcggaagcggcggaggaggctccggtgggggtggttcagggtcccattctatgagatatttttttacaagcgtgagccggcctgggaggggggagccccggtttatcgctgtggggtacgtggatgatactcaattcgtgcggttcgactctgacgccgcctcacagcgcatggagcctagggcaccctggattgaacaggagggcccggaatactgggacggcgaaacccgcaaggtaaaagcgcacagccagacgcatagggtggatctgggcaccctgcggggctgttataaccagtcagaggctggctcacacactgtacagcggatgtatggttgtgacgtcggttccgattggagatttcttcgcggctaccaccaatacgcctacgatggcaaggactacatcgcactgaaggaagatttgagatcttggaccgcggcggatatggcagcacagactaccaaacacaagtgggaagctgctcatgtggcagaacagctccgcgcctatctggagggcacttgcgtcgagtggttgcggagatacctggagaatggaaaagaaacactgcagcggaccgatgcacctaaaacacatatgacgcaccacgctgtgtccgaccacgaggcaacactccggtgttgggcactcagcttctaccctgctgaaataacgctgacctggcagcgcgacggcgaagatcagacgcaggacacagagcttgttgaaactcgccctgctggcgacggcaccttccaaaaatgggcagcagtagtcgtcccctccggacaggaacagcggtatacttgccacgtgcagcatgaaggtctccccaagcccctcactttgagatgggagccctcttctcaacccacgatccctattgttggcattatcgctggtctggtgctttttggagccgtgattactggagcagtggtggcagctgtgatgtggagacgcaagtcttctgataggaagggcggatcttattcccaggctgcgtccagtgacagcgcccaggggtcagatgtcagcctgaccgcatgcaaggtgggtggtggaggatctggcggcggcggaagcggagggggaggatccggaggaggcggctc

SEQ ID NO: 20 - protein, 494 aa, Artificial Sequence
  GCGGS+G4Sx2-hB2m-G4Sx4-HLA-A2 Y108C (G4S)4
GCGGSGGGGSGGGGSIQRTPKIQVYSRHPAENGKSNFLNCYVSGFHPSDIEVDLLKNGERIEKVEHSDLSFSKDWSFYLLYYTEFTPTEKDEYACRVNHVTLSQPKIVKWDRDMGGGGSGGGGSGGGGSGGGGSGSHSMRYFFTSVSRPGRGEPRFIAVGYVDDTQFVRFDSDAASQRMEPRAPWIEQEGPEYWDGETRKVKAHSQTHRVDLGTLRGCYNQSEAGSHTVQRMYGCDVGSDWRFLRGYHQYAYDGKDYIALKEDLRSWTAADMAAQTTKHKWEAAHVAEQLRAYLEGTCVEWLRRYLENGKETLQRTDAPKTHMTHHAVSDHEATLRCWALSFYPAEITLTWQRDGEDQTQDTELVETRPAGDGTFQKWAAVVVPSGQEQRYTCHVQHEGLPKPLTLRWEPSSQPTIPIVGIIAGLVLFGAVITGAVVAAVMWRRKSSDRKGGSYSQAASSDSAQGSDVSLTACKVGGGGSGGGGSGGGGSGGGG

SEQ ID NO: 21 - protein, 5 aa, Artificial Sequence
  G4S linker
GCGGS

SEQ ID NO: 22 - DNA, 1470 bp, Artificial Sequence
  mRORss-B2m-G4Sx4-HLA-A2
atgcacagacctagacgtcgtggaactcgtccacctccactggcactgctcgctgctctcctcctggctgcacgtggtgctgatgcaatacagcggactccaaagatccaggtgtatagtcgccaccccgcagagaatggaaagtccaacttccttaactgttatgtgagcggatttcacccttcagacatagaggtagaccttctgaaaaacggagagagaatagagaaggtagagcatagtgatctttctttttccaaggactggagcttctacctcctgtactataccgagtttacacccactgagaaggatgagtacgcatgccgcgtgaaccacgtaaccctttctcaaccaaagattgtaaaatgggacagagacatgggtggcggcggtagcggcgggggcggaagcggcggaggaggctccggtgggggtggttcagggtcccattctatgagatatttttttacaagcgtgagccggcctgggaggggggagccccggtttatcgctgtggggtacgtggatgatactcaattcgtgcggttcgactctgacgccgcctcacagcgcatggagcctagggcaccctggattgaacaggagggcccggaatactgggacggcgaaacccgcaaggtaaaagcgcacagccagacgcatagggtggatctgggcaccctgcggggctattataaccagtcagaggctggctcacacactgtacagcggatgtatggttgtgacgtcggttccgattggagatttcttcgcggctaccaccaatacgcctacgatggcaaggactacatcgcactgaaggaagatttgagatcttggaccgcggcggatatggcagcacagactaccaaacacaagtgggaagctgctcatgtggcagaacagctccgcgcctatctggagggcacttgcgtcgagtggttgcggagatacctggagaatgggaaagaaacactgcagcggaccgatgcacctaaaacacatatgacgcaccacgctgtgtccgaccacgaggcaacactccggtgttgggcactcagcttctaccctgctgaaataacgctgacctggcagcgcgacggcgaagatcagacgcaggacacagagcttgttgaaactcgccctgctggcgacggcaccttccaaaaatgggcagcagtagtcgtcccctccggacaggaacagcggtatacttgccacgtgcagcatgaaggtctccccaagcccctcactttgagatgggagccctcttctcaacccacgatccctattgttggcattatcgctggtctggtgctttttggagccgtgattactggagcagtggtggcagctgtgatgtggagacgcaagtcttctgataggaagggcggatcttattcccaggctgcgtccagtgacagcgcccaggggtcagatgtcagcctgaccgcatgcaaggtgtaa

SEQ ID NO: 23 - protein, 489 aa, Artificial Sequence
  mRORss-B2m-G4Sx4-HLA-A2
MHRPRRRGTRPPPLALLAALLLAARGADAIQRTPKIQVYSRHPAENGKSNFLNCYVSGFHPSDIEVDLLKNGERIEKVEHSDLSFSKDWSFYLLYYTEFTPTEKDEYACRVNHVTLSQPKIVKWDRDMGGGGSGGGGSGGGGSGGGGSGSHSMRYFFTSVSRPGRGEPRFIAVGYVDDTQFVRFDSDAASQRMEPRAPWIEQEGPEYWDGETRKVKAHSQTHRVDLGTLRGYYNQSEAGSHTVQRMYGCDVGSDWRFLRGYHQYAYDGKDYIALKEDLRSWTAADMAAQTTKHKWEAAHVAEQLRAYLEGTCVEWLRRYLENGKETLQRTDAPKTHMTHHAVSDHEATLRCWALSFYPAEITLTWQRDGEDQTQDTELVETRPAGDGTFQKWAAVVVPSGQEQRYTCHVQHEGLPKPLTLRWEPSSQPTIPIVGIIAGLVLFGAVITGAVVAAVMWRRKSSDRKGGSYSQAASSDSAQGSDVSLTACKV

SEQ ID NO: 24 - protein, 372 aa, Artificial Sequence
  Chimeric Human HLA-A2/Mouse H2-K
  SIGNAL (1)..(24)
MAVMAPRTLVLLLSGALALTQTWAGSHSMRYFFTSVSRPGRGEPRFIAVGYVDDTQFVRFDSDAASQRMEPRAPWIEQEGPEYWDGETRKVKAHSQTHRVDLGTLRGYYNQSEAGSHTVQRMYGCDVGSDWRFLRGYHQYAYDGKDYIALKEDLRSWTAADMAAQTTKHKWEAAHVAEQLRAYLEGTCVEWLRRYLENGKETLQRTDAPKTHMTHHAVSDHEATLRCWALSFYPAEITLTWQRDGEDQTQDTELVETRPAGDGTFQKWAAVVVPSGQEQRYTCHVQHEGLPKPLTLRWEPPPSTVSNMATVAVLVVLGAAIVTGAVVAFVMKMRRRNTGGKGGDYALAPGSQTSDLSLPDCKVMVHDPHSLA

SEQ ID NO: 25 - protein, 451 aa, Artificial Sequence
  GCGGS-G4Sx2-hB2m-G4Sx4-HLA-A*02:01 ecto (Y108C)-PADRE-myc-myc-6his
GCGGSGGGGSGGGGSIQRTPKIQVYSRHPAENGKSNFLNCYVSGFHPSDIEVDLLKNGERIEKVEHSDLSFSKDWSFYLLYYTEFTPTEKDEYACRVNHVTLSQPKIVKWDRDMGGGGSGGGGSGGGGSGGGGSGSHSMRYFFTSVSRPGRGEPRFIAVGYVDDTQFVRFDSDAASQRMEPRAPWIEQEGPEYWDGETRKVKAHSQTHRVDLGTLRGCYNQSEAGSHTVQRMYGCDVGSDWRFLRGYHQYAYDGKDYIALKEDLRSWTAADMAAQTTKHKWEAAHVAEQLRAYLEGTCVEWLRRYLENGKETLQRTDAPKTHMTHHAVSDHEATLRCWALSFYPAEITLTWQRDGEDQTQDTELVETRPAGDGTFQKWAAVVVPSGQEQRYTCHVQHEGLPKPLTLRWEPAKFVAAWTLKAAAEQKLISEEDLGGEQKLISEEDLHHHHHH

SEQ ID NO: 26 - protein, 438 aa, Artificial Sequence
  GCGGS-G4Sx2-hB2m-G4Sx4-HLA-A*02:01 ecto (Y108C)-myc-myc-6his
GCGGSGGGGSGGGGSIQRTPKIQVYSRHPAENGKSNFLNCYVSGFHPSDIEVDLLKNGERIEKVEHSDLSFSKDWSFYLLYYTEFTPTEKDEYACRVNHVTLSQPKIVKWDRDMGGGGSGGGGSGGGGSGGGGSGSHSMRYFFTSVSRPGRGEPRFIAVGYVDDTQFVRFDSDAASQRMEPRAPWIEQEGPEYWDGETRKVKAHSQTHRVDLGTLRGCYNQSEAGSHTVQRMYGCDVGSDWRFLRGYHQYAYDGKDYIALKEDLRSWTAADMAAQTTKHKWEAAHVAEQLRAYLEGTCVEWLRRYLENGKETLQRTDAPKTHMTHHAVSDHEATLRCWALSFYPAEITLTWQRDGEDQTQDTELVETRPAGDGTFQKWAAVVVPSGQEQRYTCHVQHEGLPKPLTLRWEPEQKLISEEDLGGEQKLISEEDLHHHHHH

SEQ ID NO: 27 - protein, 733 aa, Artificial Sequence
  GCGGS-G4Sx2-hB2m-G4Sx4-HLA-A*02:01 full length (Y108C)-G4Sx4-eGFP
GCGGSGGGGSGGGGSIQRTPKIQVYSRHPAENGKSNFLNCYVSGFHPSDIEVDLLKNGERIEKVEHSDLSFSKDWSFYLLYYTEFTPTEKDEYACRVNHVTLSQPKIVKWDRDMGGGGSGGGGSGGGGSGGGGSGSHSMRYFFTSVSRPGRGEPRFIAVGYVDDTQFVRFDSDAASQRMEPRAPWIEQEGPEYWDGETRKVKAHSQTHRVDLGTLRGCYNQSEAGSHTVQRMYGCDVGSDWRFLRGYHQYAYDGKDYIALKEDLRSWTAADMAAQTTKHKWEAAHVAEQLRAYLEGTCVEWLRRYLENGKETLQRTDAPKTHMTHHAVSDHEATLRCWALSFYPAEITLTWQRDGEDQTQDTELVETRPAGDGTFQKWAAVVVPSGQEQRYTCHVQHEGLPKPLTLRWEPSSQPTIPIVGIIAGLVLFGAVITGAVVAAVMWRRKSSDRKGGSYSQAASSDSAQGSDVSLTACKVGGGGSGGGGSGGGGSGGGGSVSKGEELFTGVVPILVELDGDVNGHKFSVSGEGEGDATYGKLTLKFICTTGKLPVPWPTLVTTLTYGVQCFSRYPDHMKQHDFFKSAMPEGYVQERTIFFKDDGNYKTRAEVKFEGDTLVNRIELKGIDFKEDGNILGHKLEYNYNSHNVYIMADKQKNGIKVNFKIRHNIEDGSVQLADHYQQNTPIGDGPVLLPDNHYLSTQSALSKDPNEKRDHMVLLEFVTAAGITLGMDELYK

SEQ ID NO: 28 - protein, 13 aa, Artificial Sequence
  PADRE
AKFVAAWTLKAAA

SEQ ID NO: 29 - protein, 8 aa, Homo sapiens
PCPAPPVA